European Patent Specification EP 3 701 009 B1, published December 18, 2024. Title: Display of Heterologous Molecules on Bacterial Cells and Membrane Vesicles. Applicant: Abera Bioscience AB. The sequence listing filed with the application follows.

SEQUENCE LISTING (64 sequences)

SEQ ID NO: 1 - protein, 1377 aa, Escherichia coli
MNRIYSLRYSAVARGFIAVSEFARKCVHKSVRRLCFPVLLLIPVLFSAGSLAGTVNNELGYQLFRDFAENKGMFRPGATNIAIYNKQGEFVGTLDKAAMPDFSAVDSEIGVATLINPQYIASVKHNGGYTNVSFGDGENRYNIVDRNNAPSLDFHAPRLDKLVTEVAPTAVTAQGAVAGAYLDKERYPVFYRLGSGTQYIKDSNGQLTKMGGAYSWLTGGTVGSLSSYQNGEMISTSSGLVFDYKLNGAMPIYGEAGDSGSPLFAFDTVQNKWVLVGVLTAGNGAGGRGNNWAVIPLDFIGQKFNEDNDAPVTFRTSEGGALEWSFNSSTGAGALTQGTTTYAMHGQQGNDLNAGKNLIFQGQNGQINLKDSVSQGAGSLTFRDNYTVTTSNGSTWTGAGIVVDNGVSVNWQVNGVKGDNLHKIGEGTLTVQGTGINEGGLKVGDGKVVLNQQADNKGQVQAFSSVNIASGRPTVVLTDERQVNPDTVSWGYRGGTLDVNGNSLTFHQLKAADYGAVLANNVDKRATITLDYALRADKVALNGWSESGKGTAGNLYKYNNPYTNTTDYFILKQSTYGYFPTDQSSNATWEFVGHSQGDAQKLVADRFNTAGYLFHGQLKGNLNVDNRLPEGVTGALVMDGAADISGTFTQENGRLTLQGHPVIHAYNTQSVADKLAASGDHSVLTQPTSFSQEDWENRSFTFDRLSLKNTDFGLGRNATLNTTIQADNSSVTLGDSRVFIDKNDGQGTAFTLEEGTSVATKDADKSVFNGTVNLDNQSVLNINDIFNGGIQANNSTVNISSDSAVLGNSTLTSTALNLNKGANALASQSFVSDGPVNISDATLSLNSRPDEVSHTLLPVYDYAGSWNLKGDDARLNVGPYSMLSGNINVQDKGTVTLGGEGELSPDLTLQNQMLYSLFNGYRNIWSGSLNAPDATVSMTDTQWSMNGNSTAGNMKLNRTIVGFNGGTSPFTTLTTDNLDAVQSAFVMRTDLNKADKLVINKSATGHDNSIWVNFLKKPSNKDTLDIPLVSAPEATADNLFRASTRVVGFSDVTPILSVRKEDGKKEWVLDGYQVARNDGQGKAAATFMHISYNNFITEVNNLNKRMGDLRDINGEAGTWVRLLNGSGSADGGFTDHYTLLQMGADRKHELGSMDLFTGVMATYTDTDASADLYSGKTKSWGGGFYASGLFRSGAYFDVIAKYIHNENKYDLNFAGAGKQNFRSHSLYAGAEVGYRYHLTDTTFVEPQAELVWGRLQGQTFNWNDSGMDVSMRRNSVNPLVGRTGVVSGKTFSGKDWSLTARAGLHYEFDLTDSADVHLKDAAGEHQINGRKDSRMLYGVGLNARFGDNTRLGLEVERSAFGKYNTDDAINANIRYSF

SEQ ID NO: 2 - protein, 1377 aa, Unknown Organism
MNRIYSLRYSAVARGFIAVSEFARKCVHKSVRRLCFPVLLLIPVLFSAGSLAGTVNNELGYQLFRDFAENKGMFRPGATNIAIYNKQGEFVGTLDKAAMPDFSAVDSEIGVATLINPQYIASVKHNGGYTNVSFGDGENRYNIVDRNNAPSLDFHAPRLDKLVTEVAPTAVTAQGAVAGAYLDKERYPVFYRLGSGTQYIKDSNGQLTKMGGAYSWLTGGTVGSLSSYQNGEMISTSSGLVFDYKLNGAMPIYGEAGDSGSPLFAFDTVQNKWVLVGVLTAGNGAGGRGNNWAVIPLDFIGQKFNEDNDAPVTFRTSEGGALEWSFNSSTGAGALTQGTTTYAMHGQQGNDLNAGKNLIFQGQNGQINLKDSVSQGAGSLTFRDNYTVTTSNGSTWTGAGIVVDNGVSVNWQVNGVKGDNLHKIGEGTLTVQGTGINEGGLKVGDGKVVLNQQADNKGQVQAFSSVNIASGRPTVVLTDERQVNPDTVSWGYRGGTLDVNGNSLTFHQLKAADYGAVLANNVDKRATITLDYALRADKVALNGWSESGKGTAGNLYKYNNPYTNTTDYFILKQSTYGYFPTDQSSNATWEFVGHSQGDAQKLVADRFNTAGYLFHGQLKGNLNVDNRLPEGVTGALVMDGAADISGTFTQENGRLTLQGHPVIHAYNTQSVADKLAASGDHSVLTQPTSFSQEDWENRSFTFDRLSLKNTDFGLGRNATLNTTIQADNSSVTLGDSRVFIDKNDGQGTAFTLEEGTSVATKDADKSVFNGTVNLDNQSVLNINDIFNGGIQANNSTVNISSDSAVLGNSTLTSTALNLNKGANALASQSFVSDGPVNISDATLSLNSRPDEVSHTLLPVYDYAGSWNLKGDDARLNVGPYSMLSGNINVQDKGTVTLGGEGELSPDLTLQNQMLYSLFNGYRNIWSGSLNAPDATVSMTDTQWSMNGNSTAGNMKLNRTIVGFNGGTSPFTTLTTDNLDAVQSAFVMRTDLNKADKLVINKSATGHDNSIWVNFLKKPSNKDTLDIPLVSAPEATADNLFRASTRVVGFSDVTPILSVRKEDGKKEWVLDGYQVARNDGQGKAAATFMHISYNNFITEVGSLNKRMGDLRDINGEAGTWVRLLNGSGSADGGFTDHYTLLQMGADRKHELGSMDLFTGVMATYTDTDASADLYSGKTKSWGGGFYASGLFRSGAYFDVIAKYIHNENKYDLNFAGAGKQNFRSHSLYAGAEVGYRYHLTDTTFVEPQAELVWGRLQGQTFNWNDSGMDVSMRRNSVNPLVGRTGVVSGKTFSGKDWSLTARAGLHYEFDLTDSADVHLKDAAGEHQINGRKDSRMLYGVGLNARFGDNTRLGLEVERSAFGKYNTDDAINANIRYSF

SEQ ID NO: 3 - protein, 1131 aa, Unknown Organism
MNRIYSLRYSAVARGFIAVSEFARKCVHKSVRRLCFPVLLLIPVLFSAGSLAGSSCGSGSGNDAPVTFRTSEGGALEWSFNSSTGAGALTQGTTTYAMHGQQGNDLNAGKNLIFQGQNGQINLKDSVSQGAGSLTFRDNYTVTTSNGSTWTGAGIVVDNGVSVNWQVNGVKGDNLHKIGEGTLTVQGTGINEGGLKVGDGKVVLNQQADNKGQVQAFSSVNIASGRPTVVLTDERQVNPDTVSWGYRGGTLDVNGNSLTFHQLKAADYGAVLANNVDKRATITLDYALRADKVALNGWSESGKGTAGNLYKYNNPYTNTTDYFILKQSTYGYFPTDQSSNATWEFVGHSQGDAQKLVADRFNTAGYLFHGQLKGNLNVDNRLPEGVTGALVMDGAADISGTFTQENGRLTLQGHPVIHAYNTQSVADKLAASGDHSVLTQPTSFSQEDWENRSFTFDRLSLKNTDFGLGRNATLNTTIQADNSSVTLGDSRVFIDKNDGQGTAFTLEEGTSVATKDADKSVFNGTVNLDNQSVLNINDIFNGGIQANNSTVNISSDSAVLGNSTLTSTALNLNKGANALASQSFVSDGPVNISDATLSLNSRPDEVSHTLLPVYDYAGSWNLKGDDARLNVGPYSMLSGNINVQDKGTVTLGGEGELSPDLTLQNQMLYSLFNGYRNIWSGSLNAPDATVSMTDTQWSMNGNSTAGNMKLNRTIVGFNGGTSPFTTLTTDNLDAVQSAFVMRTDLNKADKLVINKSATGHDNSIWVNFLKKPSNKDTLDIPLVSAPEATADNLFRASTRVVGFSDVTPILSVRKEDGKKEWVLDGYQVARNDGQGKAAATFMHISYNNFITEVGSLNKRMGDLRDINGEAGTWVRLLNGSGSADGGFTDHYTLLQMGADRKHELGSMDLFTGVMATYTDTDASADLYSGKTKSWGGGFYASGLFRSGAYFDVIAKYIHNENKYDLNFAGAGKQNFRSHSLYAGAEVGYRYHLTDTTFVEPQAELVWGRLQGQTFNWNDSGMDVSMRRNSVNPLVGRTGVVSGKTFSGKDWSLTARAGLHYEFDLTDSADVHLKDAAGEHQINGRKDSRMLYGVGLNARFGDNTRLGLEVERSAFGKYNTDDAINANIRYSF

SEQ ID NO: 4 - protein, 1143 aa, Unknown Organism
MNRIYSLRYSAVARGFIAVSEFARKCVHKSVRRLCFPVLLLIPVLFSAGSLAGSSAHIVMVDAYKPTKGSGSGNDAPVTFRTSEGGALEWSFNSSTGAGALTQGTTTYAMHGQQGNDLNAGKNLIFQGQNGQINLKDSVSQGAGSLTFRDNYTVTTSNGSTWTGAGIVVDNGVSVNWQVNGVKGDNLHKIGEGTLTVQGTGINEGGLKVGDGKVVLNQQADNKGQVQAFSSVNIASGRPTVVLTDERQVNPDTVSWGYRGGTLDVNGNSLTFHQLKAADYGAVLANNVDKRATITLDYALRADKVALNGWSESGKGTAGNLYKYNNPYTNTTDYFILKQSTYGYFPTDQSSNATWEFVGHSQGDAQKLVADRFNTAGYLFHGQLKGNLNVDNRLPEGVTGALVMDGAADISGTFTQENGRLTLQGHPVIHAYNTQSVADKLAASGDHSVLTQPTSFSQEDWENRSFTFDRLSLKNTDFGLGRNATLNTTIQADNSSVTLGDSRVFIDKNDGQGTAFTLEEGTSVATKDADKSVFNGTVNLDNQSVLNINDIFNGGIQANNSTVNISSDSAVLGNSTLTSTALNLNKGANALASQSFVSDGPVNISDATLSLNSRPDEVSHTLLPVYDYAGSWNLKGDDARLNVGPYSMLSGNINVQDKGTVTLGGEGELSPDLTLQNQMLYSLFNGYRNIWSGSLNAPDATVSMTDTQWSMNGNSTAGNMKLNRTIVGFNGGTSPFTTLTTDNLDAVQSAFVMRTDLNKADKLVINKSATGHDNSIWVNFLKKPSNKDTLDIPLVSAPEATADNLFRASTRVVGFSDVTPILSVRKEDGKKEWVLDGYQVARNDGQGKAAATFMHISYNNFITEVGSLNKRMGDLRDINGEAGTWVRLLNGSGSADGGFTDHYTLLQMGADRKHELGSMDLFTGVMATYTDTDASADLYSGKTKSWGGGFYASGLFRSGAYFDVIAKYIHNENKYDLNFAGAGKQNFRSHSLYAGAEVGYRYHLTDTTFVEPQAELVWGRLQGQTFNWNDSGMDVSMRRNSVNPLVGRTGVVSGKTFSGKDWSLTARAGLHYEFDLTDSADVHLKDAAGEHQINGRKDSRMLYGVGLNARFGDNTRLGLEVERSAFGKYNTDDAINANIRYSF

SEQ ID NO: 5 - protein, 1142 aa, Unknown Organism
MNRIYSLRYSAVARGFIAVSEFARKCVHKSVRRLCFPVLLLIPVLFSAGSLAGSSKLGDIEFIKVNKGSGSGNDAPVTFRTSEGGALEWSFNSSTGAGALTQGTTTYAMHGQQGNDLNAGKNLIFQGQNGQINLKDSVSQGAGSLTFRDNYTVTTSNGSTWTGAGIVVDNGVSVNWQVNGVKGDNLHKIGEGTLTVQGTGINEGGLKVGDGKVVLNQQADNKGQVQAFSSVNIASGRPTVVLTDERQVNPDTVSWGYRGGTLDVNGNSLTFHQLKAADYGAVLANNVDKRATITLDYALRADKVALNGWSESGKGTAGNLYKYNNPYTNTTDYFILKQSTYGYFPTDQSSNATWEFVGHSQGDAQKLVADRFNTAGYLFHGQLKGNLNVDNRLPEGVTGALVMDGAADISGTFTQENGRLTLQGHPVIHAYNTQSVADKLAASGDHSVLTQPTSFSQEDWENRSFTFDRLSLKNTDFGLGRNATLNTTIQADNSSVTLGDSRVFIDKNDGQGTAFTLEEGTSVATKDADKSVFNGTVNLDNQSVLNINDIFNGGIQANNSTVNISSDSAVLGNSTLTSTALNLNKGANALASQSFVSDGPVNISDATLSLNSRPDEVSHTLLPVYDYAGSWNLKGDDARLNVGPYSMLSGNINVQDKGTVTLGGEGELSPDLTLQNQMLYSLFNGYRNIWSGSLNAPDATVSMTDTQWSMNGNSTAGNMKLNRTIVGFNGGTSPFTTLTTDNLDAVQSAFVMRTDLNKADKLVINKSATGHDNSIWVNFLKKPSNKDTLDIPLVSAPEATADNLFRASTRVVGFSDVTPILSVRKEDGKKEWVLDGYQVARNDGQGKAAATFMHISYNNFITEVGSLNKRMGDLRDINGEAGTWVRLLNGSGSADGGFTDHYTLLQMGADRKHELGSMDLFTGVMATYTDTDASADLYSGKTKSWGGGFYASGLFRSGAYFDVIAKYIHNENKYDLNFAGAGKQNFRSHSLYAGAEVGYRYHLTDTTFVEPQAELVWGRLQGQTFNWNDSGMDVSMRRNSVNPLVGRTGVVSGKTFSGKDWSLTARAGLHYEFDLTDSADVHLKDAAGEHQINGRKDSRMLYGVGLNARFGDNTRLGLEVERSAFGKYNTDDAINANIRYSF

SEQ ID NO: 6 - protein, 1140 aa, Unknown Organism
MNRIYSLRYSAVARGFIAVSEFARKCVHKSVRRLCFPVLLLIPVLFSAGSLAGSSATHIKFSKRDGSGSGNDAPVTFRTSEGGALEWSFNSSTGAGALTQGTTTYAMHGQQGNDLNAGKNLIFQGQNGQINLKDSVSQGAGSLTFRDNYTVTTSNGSTWTGAGIVVDNGVSVNWQVNGVKGDNLHKIGEGTLTVQGTGINEGGLKVGDGKVVLNQQADNKGQVQAFSSVNIASGRPTVVLTDERQVNPDTVSWGYRGGTLDVNGNSLTFHQLKAADYGAVLANNVDKRATITLDYALRADKVALNGWSESGKGTAGNLYKYNNPYTNTTDYFILKQSTYGYFPTDQSSNATWEFVGHSQGDAQKLVADRFNTAGYLFHGQLKGNLNVDNRLPEGVTGALVMDGAADISGTFTQENGRLTLQGHPVIHAYNTQSVADKLAASGDHSVLTQPTSFSQEDWENRSFTFDRLSLKNTDFGLGRNATLNTTIQADNSSVTLGDSRVFIDKNDGQGTAFTLEEGTSVATKDADKSVFNGTVNLDNQSVLNINDIFNGGIQANNSTVNISSDSAVLGNSTLTSTALNLNKGANALASQSFVSDGPVNISDATLSLNSRPDEVSHTLLPVYDYAGSWNLKGDDARLNVGPYSMLSGNINVQDKGTVTLGGEGELSPDLTLQNQMLYSLFNGYRNIWSGSLNAPDATVSMTDTQWSMNGNSTAGNMKLNRTIVGFNGGTSPFTTLTTDNLDAVQSAFVMRTDLNKADKLVINKSATGHDNSIWVNFLKKPSNKDTLDIPLVSAPEATADNLFRASTRVVGFSDVTPILSVRKEDGKKEWVLDGYQVARNDGQGKAAATFMHISYNNFITEVGSLNKRMGDLRDINGEAGTWVRLLNGSGSADGGFTDHYTLLQMGADRKHELGSMDLFTGVMATYTDTDASADLYSGKTKSWGGGFYASGLFRSGAYFDVIAKYIHNENKYDLNFAGAGKQNFRSHSLYAGAEVGYRYHLTDTTFVEPQAELVWGRLQGQTFNWNDSGMDVSMRRNSVNPLVGRTGVVSGKTFSGKDWSLTARAGLHYEFDLTDSADVHLKDAAGEHQINGRKDSRMLYGVGLNARFGDNTRLGLEVERSAFGKYNTDDAINANIRYSF

SEQ ID NO: 7 - protein, 1222 aa, Unknown Organism
MNRIYSLRYSAVARGFIAVSEFARKCVHKSVRRLCFPVLLLIPVLFSAGSLAGSSDSATHIKFSKRDEDGKELAGATMELRDSSGKTISTWISDGQVKDFYLYPGKYTFVETAAPDGYEVATAITFTVNEQGQVTVNGKATKGDAHIGSGSGNDAPVTFRTSEGGALEWSFNSSTGAGALTQGTTTYAMHGQQGNDLNAGKNLIFQGQNGQINLKDSVSQGAGSLTFRDNYTVTTSNGSTWTGAGIVVDNGVSVNWQVNGVKGDNLHKIGEGTLTVQGTGINEGGLKVGDGKVVLNQQADNKGQVQAFSSVNIASGRPTVVLTDERQVNPDTVSWGYRGGTLDVNGNSLTFHQLKAADYGAVLANNVDKRATITLDYALRADKVALNGWSESGKGTAGNLYKYNNPYTNTTDYFILKQSTYGYFPTDQSSNATWEFVGHSQGDAQKLVADRFNTAGYLFHGQLKGNLNVDNRLPEGVTGALVMDGAADISGTFTQENGRLTLQGHPVIHAYNTQSVADKLAASGDHSVLTQPTSFSQEDWENRSFTFDRLSLKNTDFGLGRNATLNTTIQADNSSVTLGDSRVFIDKNDGQGTAFTLEEGTSVATKDADKSVFNGTVNLDNQSVLNINDIFNGGIQANNSTVNISSDSAVLGNSTLTSTALNLNKGANALASQSFVSDGPVNISDATLSLNSRPDEVSHTLLPVYDYAGSWNLKGDDARLNVGPYSMLSGNINVQDKGTVTLGGEGELSPDLTLQNQMLYSLFNGYRNIWSGSLNAPDATVSMTDTQWSMNGNSTAGNMKLNRTIVGFNGGTSPFTTLTTDNLDAVQSAFVMRTDLNKADKLVINKSATGHDNSIWVNFLKKPSNKDTLDIPLVSAPEATADNLFRASTRVVGFSDVTPILSVRKEDGKKEWVLDGYQVARNDGQGKAAATFMHISYNNFITEVGSLNKRMGDLRDINGEAGTWVRLLNGSGSADGGFTDHYTLLQMGADRKHELGSMDLFTGVMATYTDTDASADLYSGKTKSWGGGFYASGLFRSGAYFDVIAKYIHNENKYDLNFAGAGKQNFRSHSLYAGAEVGYRYHLTDTTFVEPQAELVWGRLQGQTFNWNDSGMDVSMRRNSVNPLVGRTGVVSGKTFSGKDWSLTARAGLHYEFDLTDSADVHLKDAAGEHQINGRKDSRMLYGVGLNARFGDNTRLGLEVERSAFGKYNTDDAINANIRYSF

SEQ ID NO: 8 - protein, 1242 aa, Unknown Organism
MNRIYSLRYSAVARGFIAVSEFARKCVHKSVRRLCFPVLLLIPVLFSAGSLAGSSKPLRGAVFSLQKQHPDYPDIYGAIDQNGTYQNVRTGEDGKLTFKNLSDGKYRLFENSEPAGYKPVQNKPIVAFQIVNGEVRDVTSIVPQDIPATYEFTNGKHYITNEPIPPKGSGSGNDAPVTFRTSEGGALEWSFNSSTGAGALTQGTTTYAMHGQQGNDLNAGKNLIFQGQNGQINLKDSVSQGAGSLTFRDNYTVTTSNGSTWTGAGIVVDNGVSVNWQVNGVKGDNLHKIGEGTLTVQGTGINEGGLKVGDGKVVLNQQADNKGQVQAFSSVNIASGRPTVVLTDERQVNPDTVSWGYRGGTLDVNGNSLTFHQLKAADYGAVLANNVDKRATITLDYALRADKVALNGWSESGKGTAGNLYKYNNPYTNTTDYFILKQSTYGYFPTDQSSNATWEFVGHSQGDAQKLVADRFNTAGYLFHGQLKGNLNVDNRLPEGVTGALVMDGAADISGTFTQENGRLTLQGHPVIHAYNTQSVADKLAASGDHSVLTQPTSFSQEDWENRSFTFDRLSLKNTDFGLGRNATLNTTIQADNSSVTLGDSRVFIDKNDGQGTAFTLEEGTSVATKDADKSVFNGTVNLDNQSVLNINDIFNGGIQANNSTVNISSDSAVLGNSTLTSTALNLNKGANALASQSFVSDGPVNISDATLSLNSRPDEVSHTLLPVYDYAGSWNLKGDDARLNVGPYSMLSGNINVQDKGTVTLGGEGELSPDLTLQNQMLYSLFNGYRNIWSGSLNAPDATVSMTDTQWSMNGNSTAGNMKLNRTIVGFNGGTSPFTTLTTDNLDAVQSAFVMRTDLNKADKLVINKSATGHDNSIWVNFLKKPSNKDTLDIPLVSAPEATADNLFRASTRVVGFSDVTPILSVRKEDGKKEWVLDGYQVARNDGQGKAAATFMHISYNNFITEVGSLNKRMGDLRDINGEAGTWVRLLNGSGSADGGFTDHYTLLQMGADRKHELGSMDLFTGVMATYTDTDASADLYSGKTKSWGGGFYASGLFRSGAYFDVIAKYIHNENKYDLNFAGAGKQNFRSHSLYAGAEVGYRYHLTDTTFVEPQAELVWGRLQGQTFNWNDSGMDVSMRRNSVNPLVGRTGVVSGKTFSGKDWSLTARAGLHYEFDLTDSADVHLKDAAGEHQINGRKDSRMLYGVGLNARFGDNTRLGLEVERSAFGKYNTDDAINANIRYSF

SEQ ID NO: 9 - protein, 1326 aa, Unknown Organism
MNRIYSLRYSAVARGFIAVSEFARKCVHKSVRRLCFPVLLLIPVLFSAGSLAGTVNNELGYQLFRDFAENKGMFRPGATNIAIYNKQGEFVGTLDKAAMPDFSAVDSEIGVATLINPQYIASVKHNGGYTNVSFGDGENRYNIVDRNNAPSLDFHAPRLDKLVTEVAPTAVTAQGAVAGAYLDKERYPVFYRLGSGTQYIKDSNGQLTKMGGAYSWLTGGTVGSLSSYQNGEMISTSSGLVFDYKLNGAMPIYGEAGDSGSPLFAFDTVQNKWVLVGVLTAGNGAGGRGNNWAVIPLDFIGQKFNEDNDAPVTFRTSEGGALEWSFNSSTGAGALTQGTTTYAMHGQQGNDLNAGKNLIFQGQNGQINLKDSVSQGAGSLTFRDNYTVTTSNGSTWTGAGIVVDNGVSVNWQVNGVKGDNLHKIGEGTLTVQGTGINEGGLKVGDGKVVLNQQADNKGQVQAFSSVNIASGRPTVVLTDERQVNPDTVSWGYRGGTLDVNGNSLTFHQLKAADYGAVLANNVDKRATITLDYAGSGSSAHIVMVDAYKPTKGSGSGNTAGYLFHGQLKGNLNVDNRLPEGVTGALVMDGAADISGTFTQENGRLTLQGHPVIHAYNTQSVADKLAASGDHSVLTQPTSFSQEDWENRSFTFDRLSLKNTDFGLGRNATLNTTIQADNSSVTLGDSRVFIDKNDGQGTAFTLEEGTSVATKDADKSVFNGTVNLDNQSVLNINDIFNGGIQANNSTVNISSDSAVLGNSTLTSTALNLNKGANALASQSFVSDGPVNISDATLSLNSRPDEVSHTLLPVYDYAGSWNLKGDDARLNVGPYSMLSGNINVQDKGTVTLGGEGELSPDLTLQNQMLYSLFNGYRNIWSGSLNAPDATVSMTDTQWSMNGNSTAGNMKLNRTIVGFNGGTSPFTTLTTDNLDAVQSAFVMRTDLNKADKLVINKSATGHDNSIWVNFLKKPSNKDTLDIPLVSAPEATADNLFRASTRVVGFSDVTPILSVRKEDGKKEWVLDGYQVARNDGQGKAAATFMHISYNNFITEVGSLNKRMGDLRDINGEAGTWVRLLNGSGSADGGFTDHYTLLQMGADRKHELGSMDLFTGVMATYTDTDASADLYSGKTKSWGGGFYASGLFRSGAYFDVIAKYIHNENKYDLNFAGAGKQNFRSHSLYAGAEVGYRYHLTDTTFVEPQAELVWGRLQGQTFNWNDSGMDVSMRRNSVNPLVGRTGVVSGKTFSGKDWSLTARAGLHYEFDLTDSADVHLKDAAGEHQINGRKDSRMLYGVGLNARFGDNTRLGLEVERSAFGKYNTDDAINANIRYSF

SEQ ID NO: 10 - protein, 1336 aa, Unknown Organism
MNRIYSLRYSAVARGFIAVSEFARKCVHKSVRRLCFPVLLLIPVLFSAGSLAGTVNNELGYQLFRDFAENKGMFRPGATNIAIYNKQGEFVGTLDKAAMPDFSAVDSEIGVATLINPQYIASVKHNGGYTNVSFGDGENRYNIVDRNNAPSLDFHAPRLDKLVTEVAPTAVTAQGAVAGAYLDKERYPVFYRLGSGTQYIKDSNGQLTKMGGAYSWLTGGTVGSLSSYQNGEMISTSSGLVFDYKLNGAMPIYGEAGDSGSPLFAFDTVQNKWVLVGVLTAGNGAGGRGNNWAVIPLDFIGQKFNEDNDAPVTFRTSEGGALEWSFNSSTGAGALTQGTTTYAMHGQQGNDLNAGKNLIFQGQNGQINLKDSVSQGAGSLTFRDNYTVTTSNGSTWTGAGIVVDNGVSVNWQVNGVKGDNLHKIGEGTLTVQGTGINEGGLKVGDGKVVLNQQADNKGQVQAFSSVNIASGRPTVVLTDERQVNPDTVSWGYRGGTLDVNGNSLTFHQLKAADYGAVLANNVDKRATITLDYAGSGSSGSASGAHIVMVDAYKPTKGEGTGGSGSGNTAGYLFHGQLKGNLNVDNRLPEGVTGALVMDGAADISGTFTQENGRLTLQGHPVIHAYNTQSVADKLAASGDHSVLTQPTSFSQEDWENRSFTFDRLSLKNTDFGLGRNATLNTTIQADNSSVTLGDSRVFIDKNDGQGTAFTLEEGTSVATKDADKSVFNGTVNLDNQSVLNINDIFNGGIQANNSTVNISSDSAVLGNSTLTSTALNLNKGANALASQSFVSDGPVNISDATLSLNSRPDEVSHTLLPVYDYAGSWNLKGDDARLNVGPYSMLSGNINVQDKGTVTLGGEGELSPDLTLQNQMLYSLFNGYRNIWSGSLNAPDATVSMTDTQWSMNGNSTAGNMKLNRTIVGFNGGTSPFTTLTTDNLDAVQSAFVMRTDLNKADKLVINKSATGHDNSIWVNFLKKPSNKDTLDIPLVSAPEATADNLFRASTRVVGFSDVTPILSVRKEDGKKEWVLDGYQVARNDGQGKAAATFMHISYNNFITEVGSLNKRMGDLRDINGEAGTWVRLLNGSGSADGGFTDHYTLLQMGADRKHELGSMDLFTGVMATYTDTDASADLYSGKTKSWGGGFYASGLFRSGAYFDVIAKYIHNENKYDLNFAGAGKQNFRSHSLYAGAEVGYRYHLTDTTFVEPQAELVWGRLQGQTFNWNDSGMDVSMRRNSVNPLVGRTGVVSGKTFSGKDWSLTARAGLHYEFDLTDSADVHLKDAAGEHQINGRKDSRMLYGVGLNARFGDNTRLGLEVERSAFGKYNTDDAINANIRYSF

SEQ ID NO: 11 - protein, 1325 aa, Unknown Organism
MNRIYSLRYSAVARGFIAVSEFARKCVHKSVRRLCFPVLLLIPVLFSAGSLAGTVNNELGYQLFRDFAENKGMFRPGATNIAIYNKQGEFVGTLDKAAMPDFSAVDSEIGVATLINPQYIASVKHNGGYTNVSFGDGENRYNIVDRNNAPSLDFHAPRLDKLVTEVAPTAVTAQGAVAGAYLDKERYPVFYRLGSGTQYIKDSNGQLTKMGGAYSWLTGGTVGSLSSYQNGEMISTSSGLVFDYKLNGAMPIYGEAGDSGSPLFAFDTVQNKWVLVGVLTAGNGAGGRGNNWAVIPLDFIGQKFNEDNDAPVTFRTSEGGALEWSFNSSTGAGALTQGTTTYAMHGQQGNDLNAGKNLIFQGQNGQINLKDSVSQGAGSLTFRDNYTVTTSNGSTWTGAGIVVDNGVSVNWQVNGVKGDNLHKIGEGTLTVQGTGINEGGLKVGDGKVVLNQQADNKGQVQAFSSVNIASGRPTVVLTDERQVNPDTVSWGYRGGTLDVNGNSLTFHQLKAADYGAVLANNVDKRATITLDYAGSGSSKLGDIEFIKVNKGSGSGNTAGYLFHGQLKGNLNVDNRLPEGVTGALVMDGAADISGTFTQENGRLTLQGHPVIHAYNTQSVADKLAASGDHSVLTQPTSFSQEDWENRSFTFDRLSLKNTDFGLGRNATLNTTIQADNSSVTLGDSRVFIDKNDGQGTAFTLEEGTSVATKDADKSVFNGTVNLDNQSVLNINDIFNGGIQANNSTVNISSDSAVLGNSTLTSTALNLNKGANALASQSFVSDGPVNISDATLSLNSRPDEVSHTLLPVYDYAGSWNLKGDDARLNVGPYSMLSGNINVQDKGTVTLGGEGELSPDLTLQNQMLYSLFNGYRNIWSGSLNAPDATVSMTDTQWSMNGNSTAGNMKLNRTIVGFNGGTSPFTTLTTDNLDAVQSAFVMRTDLNKADKLVINKSATGHDNSIWVNFLKKPSNKDTLDIPLVSAPEATADNLFRASTRVVGFSDVTPILSVRKEDGKKEWVLDGYQVARNDGQGKAAATFMHISYNNFITEVGSLNKRMGDLRDINGEAGTWVRLLNGSGSADGGFTDHYTLLQMGADRKHELGSMDLFTGVMATYTDTDASADLYSGKTKSWGGGFYASGLFRSGAYFDVIAKYIHNENKYDLNFAGAGKQNFRSHSLYAGAEVGYRYHLTDTTFVEPQAELVWGRLQGQTFNWNDSGMDVSMRRNSVNPLVGRTGVVSGKTFSGKDWSLTARAGLHYEFDLTDSADVHLKDAAGEHQINGRKDSRMLYGVGLNARFGDNTRLGLEVERSAFGKYNTDDAINANIRYSF

SEQ ID NO: 12 - protein, 1395 aa, Unknown Organism
MNRIYSLRYSAVARGFIAVSEFARKCVHKSVRRLCFPVLLLIPVLFSAGSLAGTVNNELGYQLFRDFAENKGMFRPGATNIAIYNKQGEFVGTLDKAAMPDFSAVDSEIGVATLINPQYIASVKHNGGYTNVSFGDGENRYNIVDRNNAPSLDFHAPRLDKLVTEVAPTAVTAQGAVAGAYLDKERYPVFYRLGSGTQYIKDSNGQLTKMGGAYSWLTGGTVGSLSSYQNGEMISTSSGLVFDYKLNGAMPIYGEAGDSGSPLFAFDTVQNKWVLVGVLTAGNGAGGRGNNWAVIPLDFIGQKFNEDNDAPVTFRTSEGGALEWSFNSSTGAGALTQGTTTYAMHGQQGNDLNAGKNLIFQGQNGQINLKDSVSQGAGSLTFRDNYTVTTSNGSTWTGAGIVVDNGVSVNWQVNGVKGDNLHKIGEGTLTVQGTGINEGGLKVGDGKVVLNQQADNKGQVQAFSSVNIASGRPTVVLTDERQVNPDTVSWGYRGGTLDVNGNSLTFHQLKAADYGAVLANNVDKRATITLDYALRADKVALNGWSESGKGTAGNLYKYNNPYTNTTDYFILKQSTYGYFPTDQSSNATWEFVGHSQGDAQKLVADRFNTAGYLFHGQLKGNLNVDNRLPEGVTGALVMDGAADISGTFTQENGRLTLQGHPVIHAYNTQSVADKLAASGDHSVLTQPTSFSQEDWENRSFTFDRLSLKNTDFGLGRNATLNTTIQADNSSVTLGDSRVFIDKNDGQGTAFTLEEGTSVAGSGSSAHIVMVDAYKPTKGSGSGKSVFNGTVNLDNQSVLNINDIFNGGIQANNSTVNISSDSAVLGNSTLTSTALNLNKGANALASQSFVSDGPVNISDATLSLNSRPDEVSHTLLPVYDYAGSWNLKGDDARLNVGPYSMLSGNINVQDKGTVTLGGEGELSPDLTLQNQMLYSLFNGYRNIWSGSLNAPDATVSMTDTQWSMNGNSTAGNMKLNRTIVGFNGGTSPFTTLTTDNLDAVQSAFVMRTDLNKADKLVINKSATGHDNSIWVNFLKKPSNKDTLDIPLVSAPEATADNLFRASTRVVGFSDVTPILSVRKEDGKKEWVLDGYQVARNDGQGKAAATFMHISYNNFITEVGSLNKRMGDLRDINGEAGTWVRLLNGSGSADGGFTDHYTLLQMGADRKHELGSMDLFTGVMATYTDTDASADLYSGKTKSWGGGFYASGLFRSGAYFDVIAKYIHNENKYDLNFAGAGKQNFRSHSLYAGAEVGYRYHLTDTTFVEPQAELVWGRLQGQTFNWNDSGMDVSMRRNSVNPLVGRTGVVSGKTFSGKDWSLTARAGLHYEFDLTDSADVHLKDAAGEHQINGRKDSRMLYGVGLNARFGDNTRLGLEVERSAFGKYNTDDAINANIRYSF

SEQ ID NO: 13 - protein, 1405 aa, Unknown Organism
MNRIYSLRYSAVARGFIAVSEFARKCVHKSVRRLCFPVLLLIPVLFSAGSLAGTVNNELGYQLFRDFAENKGMFRPGATNIAIYNKQGEFVGTLDKAAMPDFSAVDSEIGVATLINPQYIASVKHNGGYTNVSFGDGENRYNIVDRNNAPSLDFHAPRLDKLVTEVAPTAVTAQGAVAGAYLDKERYPVFYRLGSGTQYIKDSNGQLTKMGGAYSWLTGGTVGSLSSYQNGEMISTSSGLVFDYKLNGAMPIYGEAGDSGSPLFAFDTVQNKWVLVGVLTAGNGAGGRGNNWAVIPLDFIGQKFNEDNDAPVTFRTSEGGALEWSFNSSTGAGALTQGTTTYAMHGQQGNDLNAGKNLIFQGQNGQINLKDSVSQGAGSLTFRDNYTVTTSNGSTWTGAGIVVDNGVSVNWQVNGVKGDNLHKIGEGTLTVQGTGINEGGLKVGDGKVVLNQQADNKGQVQAFSSVNIASGRPTVVLTDERQVNPDTVSWGYRGGTLDVNGNSLTFHQLKAADYGAVLANNVDKRATITLDYALRADKVALNGWSESGKGTAGNLYKYNNPYTNTTDYFILKQSTYGYFPTDQSSNATWEFVGHSQGDAQKLVADRFNTAGYLFHGQLKGNLNVDNRLPEGVTGALVMDGAADISGTFTQENGRLTLQGHPVIHAYNTQSVADKLAASGDHSVLTQPTSFSQEDWENRSFTFDRLSLKNTDFGLGRNATLNTTIQADNSSVTLGDSRVFIDKNDGQGTAFTLEEGTSVAGSGSSGSASGAHIVMVDAYKPTKGEGTGGSGSGKSVFNGTVNLDNQSVLNINDIFNGGIQANNSTVNISSDSAVLGNSTLTSTALNLNKGANALASQSFVSDGPVNISDATLSLNSRPDEVSHTLLPVYDYAGSLNLKGDDARLNVGPYSMLSGNINVQDKGTVTLGGEGELSPDLTLQNQMLYSLFNGYRNIWSGSLNAPDATVSMTDTQWSMNGNSTAGNMKLNRTIVGFNGGTSPFTTLTTDNLDAVQSAFVMRTDLNKADKLVINKSATGHDNSIWVNFLKKPSNKDTLDIPLVSAPEATADNLFRASTRVVGFSDVTPILSVRKEDGKKEWVLDGYQVARNDGQGKAAATFMHISYNNFITEVGSLNKRMGDLRDINGEAGTWVRLLNGSGSADGGFTDHYTLLQMGADRKHELGSMDLFTGVMATYTDTDASADLYSGKTKSWGGGFYASGLFRSGAYFDVIAKYIHNENKYDLNFAGAGKQNFRSHSLYAGAEVGYRYHLTDTTFVEPQAELVWGRLQGQTFNWNDSGMDVSMRRNSVNPLVGRTGVVSGKTFSGKDWSLTARAGLHYEFDLTDSADVHLKDAAGEHQINGRKDSRMLYGVGLNARFGDNTRLGLEVERSAFGKYNTDDAINANIRYSF

SEQ ID NO: 14 - protein, 256 aa, Unknown Organism
MSYYHHHHHHDYDSATHIKFSKRDEDGKELAGATMELRDSSGKTISTWISDGQVKDFYLYPGKYTFVETAAPDGYEVATAITFTVNEQGQVTVNGKATKGDAHIGSPANLKALEAQKQKEQRQAAEELANAKKLKEQLEKGSHMKPLRGAVFSLQKQHPDYPDIYGAIDQNGTYQNVRTGEDGKLTFKNLSDGKYRLFENSEPAGYKPVQNKPIVAFQIVNGEVRDVTSIVPQDIPATYEFTNGKHYITNEPIPPK

SEQ ID NO: 15 - protein, 245 aa, Unknown Organism
MKYLLPTAAAGLLLLAAQPAMAMVQLVESGGALVQPGGSLRLSCAASGFPVNRYSMRWYRQAPGKEREWVAGMSSAGDRSSYEDSVKGRFTISRDDARNTVYLQMNSLKPEDTAVYYCNVNVGFEYWGQGTQVTVSSKGSGGTGDSATHIKFSKRDEDGKELAGATMELRDSSGKTISTWISDGQVKDFYLYPGKYTFVETAAPDGYEVATAITFTVNEQGQVTVNGKATKGDAHIGSGHHHHHH

SEQ ID NO: 16 - protein, 245 aa, Unknown Organism
MKYLLPTAAAGLLLLAAQPAMAMVQLVESGGALVQPGGSLRLSCAASGFPVNRYSMRWYRQAPGKEREWVAGMSSAGDRSSYEDSVKGRFTISRDDARNTVYLQMNSLKPEDTAVYYCNVNVGFEYWGQGTQVTVSSKGSGGTGDSATHIKFSKRDEDGKELAGATMELRDSSGKTISTWISDGQVKDFYLYPGKYTFVQTAAPDGYEVATAITFTVNEQGQVTVNGKATKGDAHIGSGHHHHHH

SEQ ID NO: 17 - protein, 356 aa, Unknown Organism
MGDSATHIKFSKRDEDGKELAGATMELRDSSGKTISTWISDGQVKDFYLYPGKYTFVETAAPDGYEVATAITFTVNEQGQVTVNGKATKGDAHIGSGYPYDVPDYAGSGEFEESPQVVEKSSLEKKYEEAKAKADTAKKDYETAKKKAEDAQKKYEDDQKRTEEKARKEAEASQKLNDVALVVQNAYKEYREVQNQRSKYKSDAEYQKKLTEVDSKIEKARKEQQDLQNKFNEVRAVVVPEPNALAETKKKAEEAKAEEKVAKRKYDYATLKVALAKKEVEAKELEIEKLQYEISTLEQEVATAQHQVDNLKKLLAGADPDDGTVDGSGGTGKLGDIEFIKVNKGSGESGHHHHHH

SEQ ID NO: 18 - protein, 782 aa, Unknown Organism
MGDSATHIKFSKRDEDGKELAGATMELRDSSGKTISTWISDGQVKDFYLYPGKYTFVETAAPDGYEVATAITFTVNEQGQVTVNGKATKGDAHIGSGYPYDVPDYAGSGEFEESPQVVEKSSLEKKYEEAKAKADTAKKDYETAKKKAEDAQKKYEDDQKRTEEKARKEAEASQKLNDVALVVQNAYKEYREVQNQRSKYKSDAEYQKKLTEVDSKIEKARKEQQDLQNKFNEVRAVVVPEPNALAETKKKAEEAKAEEKVAKRKYDYATLKVALAKKEVEAKELEIEKLQYEISTLEQEVATAQHQVDNLKKLLAGADPDDGTVEASSGKKEATTSTEPPTELSGEITMWHSFTQGPRLESIQKSADAFMQKHPKTKIKIETFSWNDFYTKWTTGLANGNVPDISTALPNQVMEMVNSDALVPLNDSIKRIGQDKFNETALNEAKIGDDYYSVPLYSHAQVMWVRTDLLKEHNIEVPKTWDQLYEASKKLKEAGVYGLSVPFGTNDLMATRFLNFYVRSGGGSLLTKDLKADLTSQLAQDGIKYWVKLYKEISPQDSLNFNVLQQATLFYQGKTAFDFNSGFHIGGINANSPQLIDSIDAYPIPKIKESDKDQGIETSNIPMVVWKNSKHPEVAKAFLEALYNEEDYVKFLDSTPVGMLPTIKGISDSAAYKENETRKKFKHAEEVITEAVKKGTAIGYENGPSVQAGMLTNQHIIEQMFQDIITNGTDPMKAAKEAEKQLNDLFEAVQVDGSGGTGKLGDIEFIKVNKGSGESGHHHHHH

SEQ ID NO: 19 - protein, 411 aa, Unknown Organism
MGSSHHHHHHSSGLVPRGSHMGAHIVMVDAYKPTKGSGESGKIEEGKLVIWINGDKGYNGLAEVGKKFEKDTGIKVTVEHPDKLEEKFPQVAATGDGPDIIFWAHDRFGGYAQSGLLAEITPDKAFQDKLYPFTWDAVRYNGKLIAYPIAVEALSLIYNKDLLPNPPKTWEEIPALDKELKAKGKSALMFNLQEPYFTWPLIAADGGYAFKYENGKYDIKDVGVDNAGAKAGLTFLVDLIKNKHMNADTDYSIAEAAFNKGETAMTINGPWAWSNIDTSKVNYGVTVLPTFKGQPSKPFVGVLSAGINAASPNKELAKEFLENYLLTDEGLEAVNKDKPLGAVALKSYEEELAKDPRIAATMENAQKGEIMPNIPQMSAFWYAVRTAVINAASGRQTVDEALKDAQTNSSS

SEQ ID NO: 20 - protein, 410 aa, Unknown Organism
MGSSHHHHHHSSGLVPRGSHMGKLGDIEFIKVNKGSGESGKIEEGKLVIWINGDKGYNGLAEVGKKFEKDTGIKVTVEHPDKLEEKFPQVAATGDGPDIIFWAHDRFGGYAQSGLLAEITPDKAFQDKLYPFTWDAVRYNGKLIAYPIAVEALSLIYNKDLLPNPPKTWEEIPALDKELKAKGKSALMFNLQEPYFTWPLIAADGGYAFKYENGKYDIKDVGVDNAGAKAGLTFLVDLIKNKHMNADTDYSIAEAAFNKGETAMTINGPWAWSNIDTSKVNYGVTVLPTFKGQPSKPFVGVLSAGINAASPNKELAKEFLENYLLTDEGLEAVNKDKPLGAVALKSYEEELAKDPRIAATMENAQKGEIMPNIPQMSAFWYAVRTAVINAASGRQTVDEALKDAQTNSSS

SEQ ID NO: 21 - protein, 305 aa, Unknown Organism
MGSSHHHHHHSSGLVPRGSHMGKLGDIEFIKVNKGSGESGSGVSKGEELFTGVVPILVELDGDVNGHKFSVSGEGEGDATYGKLTLKFICTTGKLPVPWPTLVTTLTYGVQCFSRYPDHMKQHDFFKSAMPEGYVQERTIFFKDDGNYKTRAEVKFEGDTLVNRIELKGIDFKEDGNILGHKLEYNYNSHNVYIMADKQKNGIKVNFKIRHNIEDGSVQLADHYQQNTPIGDGPVLLPDNHYLSTQSKLSKDPNEKRDHMVLLEFVTAAGITLGMDELYKGSGEGSGSGSGSAHIVMVDAYKPTK

SEQ ID NO: 22 - protein, 121 aa, Unknown Organism
MGSSHHHHHHGSDSEVNQEAKPEVKPEVKPETHINLKVSDGSSEIFFKIKKTTPLRRLMEAFAKRQGKEMDSLRFLYDGIRIQADQTPEDLDMEDNDIIEAHREQIGGGATHIKFSKRDGY

SEQ ID NO: 23 - protein, 108 aa, Unknown Organism
MSYYHHHHHHDYDGQSGDGKELAGATMELRDSSGKTISTWISDGQVKDFYLYPGKYTFVETAAPDGYEVATAITFTVNEQGQVTVNGKATKGGSGGSGGSGEDSATHI

SEQ ID NO: 24 - protein, 565 aa, Unknown Organism
MGDSATHIKFSKRDEDGKELAGATMELRDSSGKTISTWISDGQVKDFYLYPGKYTFVETAAPDGYEVATAITFTVNEQGQVTVNGKATKGDAHIGSGYPYDVPDYAGSGEFSGKKEATTSTEPPTELSGEITMWHSFTQGPRLESIQKSADAFMQKHPKTKIKIETFSWNDFYTKWTTGLANGNVPDISTALPNQVMEMVNSDALVPLNDSIKRIGQDKFNETALNEAKIGDDYYSVPLYSHAQVMWVRTDLLKEHNIEVPKTWDQLYEASKKLKEAGVYGLSVPFGTNDLMATRFLNFYVRSGGGSLLTKDLKADLTSQLAQDGIKYWVKLYKEISPQDSLNFNVLQQATLFYQGKTAFDFNSGFHIGGINANSPQLIDSIDAYPIPKIKESDKDQGIETSNIPMVVWKNSKHPEVAKAFLEALYNEEDYVKFLDSTPVGMLPTIKGISDSAAYKENETRKKFKHAEEVITEAVKKGTAIGYENGPSVQAGMLTNQHIIEQMFQDIITNGTDPMKAAKEAEKQLNDLFEAVQVDGSGGTGKLGDIEFIKVNKGSGESGHHHHHH

SEQ ID NO: 25 - protein, 589 aa, Unknown Organism
MGKPLRGAVFSLQKQHPDYPDIYGAIDQNGTYQNVRTGEDGKLTFKNLSDGKYRLFENSEPAGYKPVQNKPIVAFQIVNGEVRDVTSIVPQDIPATYEFTNGKHYITNEPIPPKGGSGGDYKDDDDKGGSGGEFSGKKEATTSTEPPTELSGEITMWHSFTQGPRLESIQKSADAFMQKHPKTKIKIETFSWNDFYTKWTTGLANGNVPDISTALPNQVMEMVNSDALVPLNDSIKRIGQDKFNETALNEAKIGDDYYSVPLYSHAQVMWVRTDLLKEHNIEVPKTWDQLYEASKKLKEAGVYGLSVPFGTNDLMATRFLNFYVRSGGGSLLTKDLKADLTSQLAQDGIKYWVKLYKEISPQDSLNFNVLQQATLFYQGKTAFDFNSGFHIGGINANSPQLIDSIDAYPIPKIKESDKDQGIETSNIPMVVWKNSKHPEVAKAFLEALYNEEDYVKFLDSTPVGMLPTIKGISDSAAYKENETRKKFKHAEEVITEAVKKGTAIGYENGPSVQAGMLTNQHIIEQMFQDIITNGTDPMKAAKEAEKQLNDLFEAVQVDGSGGTGAHIVMVDAYKPTKGSGESGHHHHHH

SEQ ID NO: 26 - protein, 251 aa, Unknown Organism
MSKGEELFTGVVPILVELDGDVNGHKFSVSGEGEGDATYGKLTLKFICTTGKLPVPWPTLVTTLTYGVQCFSRYPDHMKRHDFFKSAMPEGYVQERTISFKDDGNYKTRAEVKFEGDTLVNRIELKGIDFKEDGNILGHKLEYNYNSHNVYITADKQKNGIKANFKIRHNIEDGSVQLADHYQQNTPIGDGPVLLPDNHYLSTQSALSKDPNEKRDHMVLLEFVTAAGITHGMDELYKKLAAALEHHHHHH

SEQ ID NO: 27 - protein, 355 aa, Unknown Organism
AETTAPSVYPLAPGTALKSNSMVTLGCLVKGYFPEPVTVTWNSGALSSGVHTFPAVLQSGLYTLTSSVTVPSSTWSSQAVTCNVAHPASSTKVDKKIVPRECNPCGCTGSEVSSVFIFPPKTKDVLTITLTPKVTCVVVDISQNDPEVRFSWFIDDVEVHTAQTHAPEKQSNSTLRSVSELPIVHRDWLNGKTFACAVNSGAFPAPIEKSISKPEGTPRGPQVYTMAPPKEEMTQSQVSITCMVKGFYPPDIYTEWKMNGQPQENYKNTPPTMDTDGSYFLYSKLNVKKETWQQGNTFTCSVLHEGLHNHHTEKSLSHSPGKLPETGGGSGGSGGSGGSGGSAHIVMVDAYKPTK

SEQ ID NO: 28 - protein, 1304 aa, Unknown Organism
MNRIYSLRYSAVARGFIAVSEFARKCVHKSVRRLCFPVLLLIPVLFSAGSLAGSSTTSTEPPTELSGEITMWHSFTQGPRLESIQKSADAFMQKHPKTKIKIETFSWNDFYTKWTTGLANGNVPDISTALPNQVMEMVNSDALVPLNDSIKRIGQDKFNETALNEAKIGDDYYSVPLYSHAQVMWVRTDLLKEHNIGSGSGNDAPVTFRTSEGGALEWSFNSSTGAGALTQGTTTYAMHGQQGNDLNAGKNLIFQGQNGQINLKDSVSQGAGSLTFRDNYTVTTSNGSTWTGAGIVVDNGVSVNWQVNGVKGDNLHKIGEGTLTVQGTGINEGGLKVGDGKVVLNQQADNKGQVQAFSSVNIASGRPTVVLTDERQVNPDTVSWGYRGGTLDVNGNSLTFHQLKAADYGAVLANNVDKRATITLDYAGSGSSRTDLLKEHNIEVPKTWDQLYEASKKLKEAGVYGLSVPFGTNDLMATRFLNFYVRSGGGSLLTKDLKADLTSQLAQDGIKYWVKLYKEISPQDSLNFNGSGSGNTAGYLFHGQLKGNLNVDNRLPEGVTGALVMDGAADISGTFTQENGRLTLQGHPVIHAYNTQSVADKLAASGDHSVLTQPTSFSQEDWENRSFTFDRLSLKNTDFGLGRNATLNTTIQADNSSVTLGDSRVFIDKNDGQGTAFTLEEGTSVATKDADKSVFNGTVNLDNQSVLNINDIFNGGIQANNSTVNISSDSAVLGNSTLTSTALNLNKGANALASQSFVSDGPVNISDATLSLNSRPDEVSHTLLPVYDYAGSWNLKGDDARLNVGPYSMLSGNINVQDKGTVTLGGEGELSPDLTLQNQMLYSLFNGYRNIWSGSLNAPDATVSMTDTQWSMNGNSTAGNMKLNRTIVGFNGGTSPFTTLTTDNLDAVQSAFVMRTDLNKADKLVINKSATGHDNSIWVNFLKKPSNKDTLDIPLVSAPEATADNLFRASTRVVGFSDVTPILSVRKEDGKKEWVLDGYQVARNDGQGKAAATFMHISYNNFITEVGSLNKRMGDLRDINGEAGTWVRLLNGSGSADGGFTDHYTLLQMGADRKHELGSMDLFTGVMATYTDTDASADLYSGKTKSWGGGFYASGLFRSGAYFDVIAKYIHNENKYDLNFAGAGKQNFRSHSLYAGAEVGYRYHLTDTTFVEPQAELVWGRLQGQTFNWNDSGMDVSMRRNSVNPLVGRTGVVSGKTFSGKDWSLTARAGLHYEFDLTDSADVHLKDAAGEHQINGRKDSRMLYGVGLNARFGDNTRLGLEVERSAFGKYNTDDAINANIRYSF

SEQ ID NO: 29 - protein, 1281 aa, Unknown Organism
MNRIYSLRYSAVARGFIAVSEFARKCVHKSVRRLCFPVLLLIPVLFSAGSLAGSSISPQDSLNFNVLQQATLFYQGKTAFDFNSGFHIGGINANSPQLIDSIDAYPIPKIKESDKDQGIETSNIPMVVWKNSKHPEVAKAFLEALYNEEDYVKFLDSTPVGMLPTIKGISDSAAYKENETRKKFKHAEEVITEAGSGSGNDAPVTFRTSEGGALEWSFNSSTGAGALTQGTTTYAMHGQQGNDLNAGKNLIFQGQNGQINLKDSVSQGAGSLTFRDNYTVTTSNGSTWTGAGIVVDNGVSVNWQVNGVKGDNLHKIGEGTLTVQGTGINEGGLKVGDGKVVLNQQADNKGQVQAFSSVNIASGRPTVVLTDERQVNPDTVSWGYRGGTLDVNGNSLTFHQLKAADYGAVLANNVDKRATITLDYAGSGSSNETRKKFKHAEEVITEAVKKGTAIGYENGPSVQAGMLTNQHIIEQMFQDIITNGTDPMKAAKEAEKQLNDLFEAVQGSGSGNTAGYLFHGQLKGNLNVDNRLPEGVTGALVMDGAADISGTFTQENGRLTLQGHPVIHAYNTQSVADKLAASGDHSVLTQPTSFSQEDWENRSFTFDRLSLKNTDFGLGRNATLNTTIQADNSSVTLGDSRVFIDKNDGQGTAFTLEEGTSVATKDADKSVFNGTVNLDNQSVLNINDIFNGGIQANNSTVNISSDSAVLGNSTLTSTALNLNKGANALASQSFVSDGPVNISDATLSLNSRPDEVSHTLLPVYDYAGSWNLKGDDARLNVGPYSMLSGNINVQDKGTVTLGGEGELSPDLTLQNQMLYSLFNGYRNIWSGSLNAPDATVSMTDTQWSMNGNSTAGNMKLNRTIVGFNGGTSPFTTLTTDNLDAVQSAFVMRTDLNKADKLVINKSATGHDNSIWVNFLKKPSNKDTLDIPLVSAPEATADNLFRASTRVVGFSDVTPILSVRKEDGKKEWVLDGYQVARNDGQGKAAATFMHISYNNFITEVGSLNKRMGDLRDINGEAGTWVRLLNGSGSADGGFTDHYTLLQMGADRKHELGSMDLFTGVMATYTDTDASADLYSGKTKSWGGGFYASGLFRSGAYFDVIAKYIHNENKYDLNFAGAGKQNFRSHSLYAGAEVGYRYHLTDTTFVEPQAELVWGRLQGQTFNWNDSGMDVSMRRNSVNPLVGRTGVVSGKTFSGKDWSLTARAGLHYEFDLTDSADVHLKDAAGEHQINGRKDSRMLYGVGLNARFGDNTRLGLEVERSAFGKYNTDDAINANIRYSF

SEQ ID NO: 30 - protein, 300 aa, Unknown Organism
MKYLLPTAAAGLLLLAAQPAMAFACKTANGTAIPIGGGSANVYVNLAPAVNVGQNLVVDLSTQIFCHNDYPETITDYVTLQRGAAYGGVLSSFSGTVKYNGSSYPFPTTSETPRVVYNSRTDKPWPVALYLTPVSSAGGVAIKAGSLIAVLILRQTNNYNSDDFQFVWNIYANNDVVVPTGSGGYPYDVPDYAGSGGTGDSATHIKFSKRDEDGKELAGATMELRDSSGKTISTWISDGQVKDFYLYPGKYTFVETAAPDGYEVATAITFTVNEQGQVTVNGKATKGDAHIGSGHHHHHH

SEQ ID NO: 31 - DNA, 19 bp, Artificial sequence
  DNA primer
ggatctcgacgctctccct

SEQ ID NO: 32 - DNA, 35 bp, Artificial sequence
  DNA primer
cggtaccaccgctgcctttgctgctaacggtaacc

SEQ ID NO: 33 - DNA, 43 bp, Artificial sequence
  DNA primer
gcagcggtggtaccggcgatagtgctacccatattaaattctc

SEQ ID NO: 34 - DNA, 62 bp, Artificial sequence
  DNA primer
gcggccgcaagcttttactaatgatggtgatgatgatgaccgctgccaatatgagcgtcacc

SEQ ID NO: 35 - DNA, 28 bp, Artificial sequence
  DNA primer
gaaaatatacatttgtccaaaccgcagc

SEQ ID NO: 36 - DNA, 28 bp, Artificial sequence
  DNA primer
gctgcggtttggacaaatgtatattttc

SEQ ID NO: 37 - DNA, 86 bp, Artificial sequence
  DNA primer
cggcgcccacatcgtgatggtggacgcctacaagccgacgaagggtagtggtgaaagtggtcatcatcatcaccatcattagtaaa

SEQ ID NO: 38 - DNA, 94 bp, Artificial sequence
  DNA primer
agcttttactaatgatggtgatgatgatgaccactttcaccactacccttcgtcggcttgtaggcgtccaccatcacgatgtgggcgccggtac

SEQ ID NO: 39 - DNA, 83 bp, Artificial sequence
  DNA primer
cggcaaactgggcgatattgaatttattaaagtgaacaaaggtagtggtgaaagtggtcatcatcatcaccatcattagtaaa

SEQ ID NO: 40 - DNA, 91 bp, Artificial sequence
  DNA primer
agcttttactaatgatggtgatgatgatgaccactttcaccactacctttgttcactttaataaattcaatatcgcccagtttgccggtac

SEQ ID NO: 41 - DNA, 40 bp, Artificial sequence
  DNA primer
atatatccatgggcgatagtgctacccatattaaattctc

SEQ ID NO: 42 - DNA, 77 bp, Artificial sequence
  DNA primer
atatatgaattcgccggaccccgcatagtcaggaacatcgtatgggtatcccgaaccaatatgagcgtcacctttag

SEQ ID NO: 43 - DNA, 27 bp, Artificial sequence
  DNA primer
atatatgtcgacggcagcggtggtacc

SEQ ID NO: 44 - DNA, 19 bp, Artificial sequence
  DNA primer
gctagttattgctcagcgg

SEQ ID NO: 45 - DNA, 28 bp, Artificial sequence
  DNA primer
atatatccatgggcaagccgctgcgtgg

SEQ ID NO: 46 - DNA, 81 bp, Artificial sequence
  DNA primer
atatatgaattccccgccgctaccgcctttatcgtcatcatccttatagtcaccgccgctaccgcctttcggcggtatcgg

SEQ ID NO: 47 - DNA, 27 bp, Artificial sequence
  DNA primer
atatatgtcgacggcagcggtggtacc

SEQ ID NO: 48 - DNA, 31 bp, Artificial sequence
  DNA primer
atatatgaattcgaagaaagtccgcaggttg

SEQ ID NO: 49 - DNA, 27 bp, Artificial sequence
  DNA primer
atatatgtcgacggtgccatcatccgg

SEQ ID NO: 50 - DNA, 41 bp, Artificial sequence
  DNA primer
atatatgaattctcaggaaaaaaagaagctacaactagtac

SEQ ID NO: 51 - DNA, 42 bp, Artificial sequence
  DNA primer
atatatgtcgacctgaacagcctcaaataaatcatttaattg

SEQ ID NO: 52 - DNA, 45 bp, Artificial sequence
  DNA primer
ggaagtcttgcggggagctccgatagtgctacccatattaaattc

SEQ ID NO: 53 - DNA, 39 bp, Artificial sequence
  DNA primer
taccgctgccggatccaatatgagcgtcacctttagttg

SEQ ID NO: 54 - DNA, 39 bp, Artificial sequence
  DNA primer
ggaagtcttgcggggagctccaagccgctgcgtggtgcc

SEQ ID NO: 55 - DNA, 38 bp, Artificial sequence
  DNA primer
taccgctgccggatcctttcggcggtatcggttcattg

SEQ ID NO: 56 - DNA, 25 bp, Artificial sequence
  DNA primer
ttgctaactttctagattacaaaac

SEQ ID NO: 57 - DNA, 75 bp, Artificial sequence
  DNA primer
taccgctgccggatcccttcgtcggcttgtaggcgtccaccatcacgatgtgggcggagctccccgcaagacttc

SEQ ID NO: 58 - DNA, 66 bp, Artificial sequence
  DNA primer
taccgctgccggatccatcacgttttgagaatttaatatgggtagcggagctccccgcaagacttc

SEQ ID NO: 59 - DNA, 39 bp, Artificial sequence
  DNA primer
ccaaactgggcgatattgaatttattaaagtgaacaaag

SEQ ID NO: 60 - DNA, 47 bp, Artificial sequence
  DNA primer
gatcctttgttcactttaataaattcaatatcgcccagtttggagct

SEQ ID NO: 61 - DNA, 42 bp, Artificial sequence
  DNA primer
ccgcccacatcgtgatggtggacgcctacaagccgacgaagg

SEQ ID NO: 62 - DNA, 50 bp, Artificial sequence
  DNA primer
gatcccttcgtcggcttgtaggcgtccaccatcacgatgtgggcggagct

SEQ ID NO: 63 - DNA, 72 bp, Artificial sequence
  DNA primer
ccggctcggctagcggtgcccacatcgtgatggtggacgcctacaagccgacgaagggtgagggaaccggcg

SEQ ID NO: 64 - DNA, 80 bp, Artificial sequence
  DNA primer
gatccgccggttccctcacccttcgtcggcttgtaggcgtccaccatcacgatgtgggcaccgctagccgagccggagct